European Patent Application EP 4 155 419 A1, published March 29, 2023. Title: MEANS AND METHOD FOR FLUORESCENT IN SITU HYBRIDIZATION USING CRISPR-CAS9 VARIANTS AND A NUCLEASE. Applicant: PixelBiotech GmbH. The sequence listing filed with the application follows.

SEQUENCE LISTING (76 sequences)

SEQ ID NO: 1 - DNA, 65 bp, artificial
  Oligo DNA template for sgRNA in Telomere
ttctaatacgactcactatagggatgaatataagggtaagggtaagggtaagttttagagctaga

SEQ ID NO: 2 - DNA, 64 bp, artificial
  Oligo DNA template for sgRNA in alpha satellite
ttctaatacgactcactatagggatgaatactttttgtagaatctgcaaggttttagagctaga

SEQ ID NO: 3 - DNA, 64 bp, artificial
  Oligo DNA template for sgRNA in MUC4 intron 1
ttctaatacgactcactatagggatgaatagcgatgtctggaaggatccagttttagagctaga

SEQ ID NO: 4 - DNA, 64 bp, artificial
  Oligo DNA template for sgRNA in MUC4 intron 1
ttctaatacgactcactatagggatgaataggtgagacgcagacaaactggttttagagctaga

SEQ ID NO: 5 - DNA, 64 bp, artificial
  Oligo DNA template for sgRNA in MUC4 intron 1
ttctaatacgactcactatagggatgaatattgggtcacggccttgcctggttttagagctaga

SEQ ID NO: 6 - DNA, 64 bp, artificial
  Oligo DNA template for sgRNA in MUC4 intron 1
ttctaatacgactcactatagggatgaatactggggtccagagttcaagcgttttagagctaga

SEQ ID NO: 7 - DNA, 64 bp, artificial
  Oligo DNA template for sgRNA in MUC4 intron 1
ttctaatacgactcactatagggatgaatacaggactaggctgagggcaagttttagagctaga

SEQ ID NO: 8 - DNA, 64 bp, artificial
  Oligo DNA template for sgRNA in MUC4 intron 1
ttctaatacgactcactatagggatgaatagaggctggggcttggggcgcgttttagagctaga

SEQ ID NO: 9 - DNA, 64 bp, artificial
  Oligo DNA template for sgRNA in MUC4 intron 1
ttctaatacgactcactatagggatgaataaagctgagcccaaatgtgctgttttagagctaga

SEQ ID NO: 10 - DNA, 64 bp, artificial
  Oligo DNA template for sgRNA in MUC4 intron 1
ttctaatacgactcactatagggatgaatactgagtcctttgcgtcgctagttttagagctaga

SEQ ID NO: 11 - DNA, 64 bp, artificial
  Oligo DNA template for sgRNA in MUC4 intron 1
ttctaatacgactcactatagggatgaataacctgcctatacttgagtctgttttagagctaga

SEQ ID NO: 12 - DNA, 64 bp, artificial
  Oligo DNA template for sgRNA in MUC4 intron 1
ttctaatacgactcactatagggatgaatagatggaaatttggtgtctacgttttagagctaga

SEQ ID NO: 13 - DNA, 30 bp, artificial
  HuluFISH probe sequence for Telomere
ttagggttagggttagggttagggttaggg

SEQ ID NO: 14 - DNA, 21 bp, artificial
  HuluFISH probe sequence for alpha satellite DNA
ctcacagagttgaaccttcct

SEQ ID NO: 15 - DNA, 18 bp, artificial
  HuluFISH probe MUC4 intron 1
cccaggcttactcgcaga

SEQ ID NO: 16 - DNA, 18 bp, artificial
  HuluFISH probe MUC4 intron 1
gagaaagacaggcagagc

SEQ ID NO: 17 - DNA, 21 bp, artificial
  HuluFISH probe MUC4 intron 1
cagagcaagaggaacagagtc

SEQ ID NO: 18 - DNA, 20 bp, artificial
  HuluFISH probe MUC4 intron 1
aaggagaaagatgtacaccc

SEQ ID NO: 19 - DNA, 19 bp, artificial
  HuluFISH probe MUC4 intron 1
ttgtgtacagagctggggg

SEQ ID NO: 20 - DNA, 20 bp, artificial
  HuluFISH probe MUC4 intron 1
tagaggggatgccaggaaag

SEQ ID NO: 21 - DNA, 20 bp, artificial
  HuluFISH probe MUC4 intron 1
ctgggtgatggagacggaag

SEQ ID NO: 22 - DNA, 21 bp, artificial
  HuluFISH probe MUC4 intron 1
aactcatgtaaagctgcaggg

SEQ ID NO: 23 - DNA, 19 bp, artificial
  HuluFISH probe MUC4 intron 1
aggaccctgggaatggaga

SEQ ID NO: 24 - DNA, 17 bp, artificial
  HuluFISH probe MUC4 intron 1
gaggagaagatcgggag

SEQ ID NO: 25 - DNA, 17 bp, artificial
  HuluFISH probe MUC4 intron 1
cagcaagcaagggaagc

SEQ ID NO: 26 - DNA, 18 bp, artificial
  HuluFISH probe MUC4 intron 1
acaaggaggagaggggca

SEQ ID NO: 27 - DNA, 20 bp, artificial
  HuluFISH probe MUC4 intron 1
ccgtgggcttcttacctctg

SEQ ID NO: 28 - DNA, 17 bp, artificial
  HuluFISH probe MUC4 intron 1
agctcgggtttaaaagc

SEQ ID NO: 29 - DNA, 21 bp, artificial
  HuluFISH probe MUC4 intron 1
ccttgggctcctccgtgtaca

SEQ ID NO: 30 - DNA, 20 bp, artificial
  HuluFISH probe MUC4 intron 1
ccaggcctgtgggagatgtt

SEQ ID NO: 31 - DNA, 21 bp, artificial
  HuluFISH probe MUC4 intron 1
cccgtcctcttccccacactt

SEQ ID NO: 32 - DNA, 18 bp, artificial
  HuluFISH probe MUC4 intron 1
gctgtccctctggcttca

SEQ ID NO: 33 - DNA, 20 bp, artificial
  HuluFISH probe MUC4 intron 1
attctgtgtttctgggtgtc

SEQ ID NO: 34 - DNA, 19 bp, artificial
  HuluFISH probe MUC4 intron 1
tgagtctttgggggagagt

SEQ ID NO: 35 - DNA, 21 bp, artificial
  HuluFISH probe MUC4 intron 1
tggggttagagtctcagctcc

SEQ ID NO: 36 - DNA, 21 bp, artificial
  HuluFISH probe MUC4 intron 1
cctctcagcaggctaagaaca

SEQ ID NO: 37 - DNA, 21 bp, artificial
  HuluFISH probe MUC4 intron 1
gtcgccgagggaaaatatttc

SEQ ID NO: 38 - DNA, 20 bp, artificial
  HuluFISH probe MUC4 intron 1
ttgggcgcatatttgaggag

SEQ ID NO: 39 - DNA, 20 bp, artificial
  HuluFISH probe MUC4 intron 1
cttcctgggagtgagtcaga

SEQ ID NO: 40 - DNA, 17 bp, artificial
  HuluFISH probe MUC4 intron 1
cgagtgccgtttaaagg

SEQ ID NO: 41 - DNA, 20 bp, artificial
  HuluFISH probe MUC4 intron 1
ctgcaagagaagccatgctg

SEQ ID NO: 42 - DNA, 19 bp, artificial
  HuluFISH probe MUC4 intron 1
ccttccacctcgggatgtt

SEQ ID NO: 43 - DNA, 18 bp, artificial
  HuluFISH probe MUC4 intron 1
gctccagtgctcatccca

SEQ ID NO: 44 - DNA, 19 bp, artificial
  HuluFISH probe MUC4 intron 1
tgccctgcagatgtggttg

SEQ ID NO: 45 - DNA, 19 bp, artificial
  HuluFISH probe MUC4 intron 1
ggagtctccacgggaatca

SEQ ID NO: 46 - DNA, 20 bp, artificial
  HuluFISH probe MUC4 intron 1
cggggaggcagcttggattt

SEQ ID NO: 47 - DNA, 18 bp, artificial
  HuluFISH probe MUC4 intron 1
ccccagggccaagtcttt

SEQ ID NO: 48 - DNA, 17 bp, artificial
  HuluFISH probe MUC4 intron 1
gccgtgaactgttctgg

SEQ ID NO: 49 - DNA, 21 bp, artificial
  HuluFISH probe MUC4 intron 1
gccccggtcccctgtgtaaaa

SEQ ID NO: 50 - DNA, 19 bp, artificial
  HuluFISH probe MUC4 intron 1
agcagtggtgaacggttgg

SEQ ID NO: 51 - DNA, 19 bp, artificial
  HuluFISH probe MUC4 intron 1
acctcctgacgcccaagtt

SEQ ID NO: 52 - DNA, 20 bp, artificial
  HuluFISH probe MUC4 intron 1
ctggacactcagctccatgt

SEQ ID NO: 53 - DNA, 20 bp, artificial
  HuluFISH probe MUC4 intron 1
caggaagtggggtctgtgga

SEQ ID NO: 54 - DNA, 21 bp, artificial
  HuluFISH probe MUC4 intron 1
acctggggtgggcgtggaaaa

SEQ ID NO: 55 - DNA, 21 bp, artificial
  HuluFISH probe MUC4 intron 1
cgtgacccggagaaggagtga

SEQ ID NO: 56 - DNA, 20 bp, artificial
  HuluFISH probe MUC4 intron 1
aggactgttggtgtgcaagg

SEQ ID NO: 57 - DNA, 19 bp, artificial
  HuluFISH probe MUC4 intron 1
gtctccatgacgacccgaa

SEQ ID NO: 58 - DNA, 20 bp, artificial
  HuluFISH probe MUC4 intron 1
gaagctaggcatgtcgtgga

SEQ ID NO: 59 - DNA, 21 bp, artificial
  HuluFISH probe MUC4 intron 1
aagtggagctgggccaggaga

SEQ ID NO: 60 - DNA, 21 bp, artificial
  HuluFISH probe MUC4 intron 1
gagatggtcgtggctgggaga

SEQ ID NO: 61 - DNA, 19 bp, artificial
  HuluFISH probe MUC4 intron 1
tggcacccacacatctgac

SEQ ID NO: 62 - DNA, 21 bp, artificial
  HuluFISH probe MUC4 intron 1
cttggcaggaaaagcagtcac

SEQ ID NO: 63 - DNA, 21 bp, artificial
  HuluFISH probe MUC4 intron 1
ccagccagccccgttcctttt

SEQ ID NO: 64 - DNA, 20 bp, artificial
  HuluFISH probe MUC4 intron 1
cctgaaggggtttacagatg

SEQ ID NO: 65 - DNA, 20 bp, artificial
  HuluFISH probe MUC4 intron 1
agggtctgtttgcacacttg

SEQ ID NO: 66 - DNA, 20 bp, artificial
  HuluFISH probe MUC4 intron 1
ccaggctgggtcacactgaa

SEQ ID NO: 67 - DNA, 19 bp, artificial
  HuluFISH probe MUC4 intron 1
gcccaggccagaggaaaaa

SEQ ID NO: 68 - DNA, 18 bp, artificial
  HuluFISH probe MUC4 intron 1
cacagggtttccacaaag

SEQ ID NO: 69 - DNA, 19 bp, artificial
  HuluFISH probe MUC4 intron 1
gctgccgcaatgagggttt

SEQ ID NO: 70 - DNA, 20 bp, artificial
  HuluFISH probe MUC4 intron 1
ccttaaggaacagccctggc

SEQ ID NO: 71 - DNA, 20 bp, artificial
  HuluFISH probe MUC4 intron 1
caagggttaaaggataaggc

SEQ ID NO: 72 - DNA, 20 bp, artificial
  HuluFISH probe MUC4 intron 1
cagcagacagaggtgggcta

SEQ ID NO: 73 - DNA, 19 bp, artificial
  HuluFISH probe MUC4 intron 1
caggcaggaatgactcaga

SEQ ID NO: 74 - DNA, 21 bp, artificial
  HuluFISH probe MUC4 intron 1
ccgtcctggttccatgccaca

SEQ ID NO: 75 - DNA, 20 bp, artificial
  HuluFISH probe MUC4 intron 1
ggcaactgggtcgaaatagg

SEQ ID NO: 76 - DNA, 21 bp, artificial
  HuluFISH probe MUC4 intron 1
ccttggtctccagcactatca